European Patent Application EP 4 752 153 A1, published June 3, 2026. Title: Novel Peptide Having Activity of Improving Skin Condition and Uses Thereof. Applicant: CAREGEN CO., LTD. Application KR. The sequence listing filed with the application follows.

SEQUENCE LISTING (23 sequences)

SEQ ID NO: 1 - protein, 8 aa, synthetic construct
EIVRKKPI

SEQ ID NO: 2 - DNA, 20 bp, synthetic construct
  source 1..20: mol_type = other DNA
caccctcaagagcctgagtc

SEQ ID NO: 3 - DNA, 20 bp, synthetic construct
  source 1..20: mol_type = other DNA
agacggctgagtagggaaca

SEQ ID NO: 4 - DNA, 20 bp, synthetic construct
  source 1..20: mol_type = other DNA
ccaggaaccgagtacaccat

SEQ ID NO: 5 - DNA, 20 bp, synthetic construct
  source 1..20: mol_type = other DNA
atacccaggttgggtgatga

SEQ ID NO: 6 - DNA, 20 bp, synthetic construct
  source 1..20: mol_type = other DNA
gcaagacctggctttggact

SEQ ID NO: 7 - DNA, 21 bp, synthetic construct
  source 1..21: mol_type = other DNA
gggagtttctggttagggctg

SEQ ID NO: 8 - DNA, 20 bp, synthetic construct
  source 1..20: mol_type = other DNA
ccttcttgggtgctggaata

SEQ ID NO: 9 - DNA, 20 bp, synthetic construct
  source 1..20: mol_type = other DNA
acacgataagggaggctgtg

SEQ ID NO: 10 - DNA, 20 bp, synthetic construct
  source 1..20: mol_type = other DNA
tcagtggctggaacagtgag

SEQ ID NO: 11 - DNA, 20 bp, synthetic construct
  source 1..20: mol_type = other DNA
tctggcatgtcccactatca

SEQ ID NO: 12 - DNA, 21 bp, synthetic construct
  source 1..21: mol_type = other DNA
ctgactttgctggagatctgg

SEQ ID NO: 13 - DNA, 20 bp, synthetic construct
  source 1..20: mol_type = other DNA
taggccatcccttgcagtag

SEQ ID NO: 14 - DNA, 18 bp, synthetic construct
  source 1..18: mol_type = other DNA
cgccgcgcggaaaagatg

SEQ ID NO: 15 - DNA, 20 bp, synthetic construct
  source 1..20: mol_type = other DNA
aaacaccagcagccgtgtaa

SEQ ID NO: 16 - DNA, 19 bp, synthetic construct
  source 1..19: mol_type = other DNA
cgaggtaggtccaggacgg

SEQ ID NO: 17 - DNA, 20 bp, synthetic construct
  source 1..20: mol_type = other DNA
ggctccttcagcttctcagg

SEQ ID NO: 18 - DNA, 20 bp, synthetic construct
  source 1..20: mol_type = other DNA
aaaagggtgttgggagggtg

SEQ ID NO: 19 - DNA, 20 bp, synthetic construct
  source 1..20: mol_type = other DNA
gaatcccattgctttggcac

SEQ ID NO: 20 - DNA, 20 bp, synthetic construct
  source 1..20: mol_type = other DNA
cacctcatcaaggcccagag

SEQ ID NO: 21 - DNA, 20 bp, synthetic construct
  source 1..20: mol_type = other DNA
agctggaggtgaagttgtcg

SEQ ID NO: 22 - DNA, 20 bp, synthetic construct
  source 1..20: mol_type = other DNA
ggagccaaaagggtcatcat

SEQ ID NO: 23 - DNA, 20 bp, synthetic construct
  source 1..20: mol_type = other DNA
gtgatggcatggactgtggt